European Patent Application EP 4 163 372 A1, published April 12, 2023. Title: Nucleic acid molecule with improved stability and use thereof. Applicant: Imnewrun Biosciences, Inc. The sequence listing filed with the application follows.

SEQUENCE LISTING (33 sequences)

SEQ ID NO: 1 - RNA, 23 nt, Artificial Sequence
  (+GC)siGFP_SS
cgccccgaccacaugaagcagca

SEQ ID NO: 2 - RNA, 23 nt, Artificial Sequence
  (+GC)siGFP_AS
gcggggcugguguacuucgucgu

SEQ ID NO: 3 - RNA, 30 nt, Artificial Sequence
  PNA-(+GC)siGFP_SS
uaacggccgccccgaccacaugaagcagca

SEQ ID NO: 4 - RNA, 30 nt, Artificial Sequence
  PNA-(+GC)siGFP_PNA+AS
attgccggcggggcugguguacuucgucgu

SEQ ID NO: 5 - RNA, 30 nt, Artificial Sequence
  PNA-(+UA)siGFP_SS
uaacggcauccccgaccacaugaagcagca

SEQ ID NO: 6 - RNA, 30 nt, Artificial Sequence
  PNA-(+UA)siGFP_PNA+AS
attgccguaggggcugguguacuucgucgu

SEQ ID NO: 7 - RNA, 30 nt, Artificial Sequence
  PNA-(+GC)siGFP_SS
cggcaaucgccccgaccacaugaagcagca

SEQ ID NO: 8 - RNA, 30 nt, Artificial Sequence
  PNA-(+GC)siGFP_PNA+AS
gccgttagcggggcugguguacuucgucgu

SEQ ID NO: 9 - RNA, 30 nt, Artificial Sequence
  PNA-(+UA)siGFP_SS
cggcaauauccccgaccacaugaagcagca

SEQ ID NO: 10 - RNA, 30 nt, Artificial Sequence
  PNA-(+UA)siGFP_PNA+AS
gccgttauaggggcugguguacuucgucgu

SEQ ID NO: 11 - RNA, 23 nt, Artificial Sequence
  siGFP(+CG)_SS
ccccgaccacaugaagcagcagc

SEQ ID NO: 12 - RNA, 23 nt, Artificial Sequence
  siGFP(+CG)_AS
ggggcugguguacuucgucgucg

SEQ ID NO: 13 - RNA, 30 nt, Artificial Sequence
  siGFP(+CG)-PNA_SS
ccccgaccacaugaagcagcagccggcaau

SEQ ID NO: 14 - RNA, 30 nt, Artificial Sequence
  siGFP(+CG)-PNA_AS+PNA
ggggcugguguacuucgucgucggccgtta

SEQ ID NO: 15 - RNA, 30 nt, Artificial Sequence
  siGFP(+AU)-PNA_SS
ccccgaccacaugaagcagcauauagcaau

SEQ ID NO: 16 - RNA, 30 nt, Artificial Sequence
  siGFP(+AU)-PNA_AS+PNA
ggggcugguguacuucgucguauatcgtta

SEQ ID NO: 17 - RNA, 28 nt, Artificial Sequence
  PNA-(+GC)siGFP_SS
uaggccgccccgaccacaugaagcagca

SEQ ID NO: 18 - RNA, 28 nt, Artificial Sequence
  PNA-(+GC)siGFP_PNA+AS
atggcgcggggcugguguacuucgucgu

SEQ ID NO: 19 - RNA, 33 nt, Artificial Sequence
  PNA-(+GC)siGFP_SS
uaauaacggccgccccgaccacaugaagcagca

SEQ ID NO: 20 - RNA, 33 nt, Artificial Sequence
  PNA-(+GC)siGFP_PNA+AS
attattgccggcggggcugguguacuucgucgu

SEQ ID NO: 21 - RNA, 22 nt, Artificial Sequence
  (+U)siGFP_SS
accccgaccacaugaagcagca

SEQ ID NO: 22 - RNA, 22 nt, Artificial Sequence
  (+U)siGFP_AS
uggggcugguguacuucgucgu

SEQ ID NO: 23 - RNA, 29 nt, Artificial Sequence
  PNA-(+U)siGFP_SS
uaacggcaccccgaccacaugaagcagca

SEQ ID NO: 24 - RNA, 29 nt, Artificial Sequence
  PNA-(+U)siGFP_PNA+AS
attgccguggggcugguguacuucgucgu

SEQ ID NO: 25 - RNA, 29 nt, Artificial Sequence
  (+U)siGFP-PNA_SS
ccccgaccacaugaagcagcaacggcaau

SEQ ID NO: 26 - RNA, 29 nt, Artificial Sequence
  (+U)siGFP-PNA_AS+PNA
ggggcugguguacuucgucguugccgtta

SEQ ID NO: 27 - protein, 22 aa, Artificial Sequence
  dNP2
KIKKVKKKGRKKIKKVKKKGRK

SEQ ID NO: 28 - protein, 9 aa, Artificial Sequence
  Tat
RKKRRQRRR

SEQ ID NO: 29 - protein, 21 aa, Artificial Sequence
  Pep-1
KETWWETWWTEWSQPKKKRKV

SEQ ID NO: 30 - protein, 27 aa, Artificial Sequence
  MPG
GLAFLGFLGAAGSTMGAWSQPKKKRKV

SEQ ID NO: 31 - protein, 16 aa, Artificial Sequence
  Penetratin
RQIKIWFQNRRMKWKK

SEQ ID NO: 32 - protein, 30 aa, Artificial Sequence
  KALA
WEAKLAKALAKALAKHLAKALAKALKACEA

SEQ ID NO: 33 - protein, 20 aa, Artificial Sequence
  CADY
GLWRALWRLLRSLWRLLWRA